European Patent Application EP 4 194 469 A1, published June 14, 2023. Title: Anti-Met Fab-Fc for the treatment of a tumor and/or metastasis. Applicant: Vertical Bio AG. Application EP. The sequence listing filed with the application follows.

SEQUENCE LISTING (43 sequences)

SEQ ID NO: 1 - protein, 10 aa, synthetic construct
  REGION 1..10: note = VL-CDR1
QSVDYDGGSY

SEQ ID NO: 2 - skipped

SEQ ID NO: 3 - protein, 9 aa, synthetic construct
  REGION 1..9: note = VL-CDR3
QQSYEDPLT

SEQ ID NO: 4 - protein, 8 aa, synthetic construct
  REGION 1..8: note = VH-CDR1
GYTFTSYW

SEQ ID NO: 5 - protein, 8 aa, synthetic construct
  REGION 1..8: note = VH-CDR2
INPSSGRT

SEQ ID NO: 6 - protein, 5 aa, synthetic construct
  REGION 1..5: note = VH-CDR3
ASRGY

SEQ ID NO: 7 - protein, 131 aa, synthetic construct
  REGION 1..131: note = humanized VL-cl03E08
METDTILLWVLLLWVPGSTGDIVLTQSPDSLAVSLGQRATINCKASQSVDYDGGSYMSWFQQKPGQPPKLLIYAASNLESGVPARFSGSGSGTDFTLTISSLQAEDVATYYCQQSYEDPLTFGGGTKVEIK

SEQ ID NO: 8 - protein, 131 aa, synthetic construct
  REGION 1..131: note = humanized VH-cl03E08
MGWSYIILFLVATATDGHSQVQLQQSGAEVKKPGASVKLSCKASGYTFTSYWIHWVRQAPGQGLEWIGEINPSSGRTNYNEKFKNRVTVTVDKSTSTAYMELSSLTSEDSAVYYCASRGYWGQGTTLTVSS

SEQ ID NO: 9 - protein, 107 aa, Homo sapiens [sequence omitted]

SEQ ID NO: 10 - protein, 98 aa, Homo sapiens
ASTKGPSVFPLAPSSKSTSGGTAALGCLVKDYFPEPVTVSWNSGALTSGVHTFPAVLQSSGLYSLSSVVTVPSSSLGTQTYICNVNHKPSNTKVDKKV

SEQ ID NO: 11 - protein, 232 aa, synthetic construct
  REGION 1..232: note = First Fc (Knob mutation)
EPKSCDKTHTCPPCPAPELLGGPSVFLFPPKPKDTLMISRTPEVTCVVVDVSHEDPEVKFNWYVDGVEVHNAKTKPREEQYNSTYRVVSVLTVLHQDWLNGKEYKCKVSNKALPAPIEKTISKAKGQPREPQVYTLPPSRDELTKNQVSLWCLVKGFYPSDIAVEWESNGQPENNYKTTPPVLDSDGSFFLYSKLTVDKSRWQQGNVFSCSVMHEALHNHYTQKSLSLSPGK

SEQ ID NO: 12 - protein, 246 aa, synthetic construct
  REGION 1..246: note = Second Fc (Hole mutations)
MGWSYIILFLVATATDGHSDKTHTCPPCPAPELLGGPSVFLFPPKPKDTLMISRTPEVTCVVVDVSHEDPEVKFNWYVDGVEVHNAKTKPREEQYNSTYRVVSVLTVLHQDWLNGKEYKCKVSNKALPAPIEKTISKAKGQPREPQVYTLPPSRDELTKNQVSLSCAVKGFYPSDIAVEWESNGQPENNYKTTPPVLDSDGSFFLVSKLTVDKSRWQQGNVFSCSVMHEALHNHYTQKSLSLSPGK

SEQ ID NO: 13 - protein, 976 aa, synthetic construct
  REGION 1..976: note = Decoy Met wt-TAGs
MKAPAVLAPGILVLLFTLVQRSNGECKEALAKSEMNVNMKYQLPNFTAETPIQNVILHEHHIFLGATNYIYVLNEEDLQKVAEYKTGPVLEHPDCFPCQDCSSKANLSGGVWKDNINMALVVDTYYDDQLISCGSVNRGTCQRHVFPHNHTADIQSEVHCIFSPQIEEPSQCPDCVVSALGAKVLSSVKDRFINFFVGNTINSSYFPDHPLHSISVRRLKETKDGFMFLTDQSYIDVLPEFRDSYPIKYVHAFESNNFIYFLTVQRETLDAQTFHTRIIRFCSINSGLHSYMEMPLECILTEKRKKRSTKKEVFNILQAAYVSKPGAQLARQIGASLNDDILFGVFAQSKPDSAEPMDRSAMCAFPIKYVNDFFNKIVNKNNVRCLQHFYGPNHEHCFNRTLLRNSSGCEARRDEYRTEFTTALQRVDLFMGQFSEVLLTSISTFIKGDLTIANLGTSEGRFMQVVVSRSGPSTPHVNFLLDSHPVSPEVIVEHTLNQNGYTLVITGKKITKIPLNGLGCRHFQSCSQCLSAPPFVQCGWCHDKCVRSEECLSGTWTQQICLPAIYKVFPNSAPLEGGTRLTICGWDFGFRRNNKFDLKKTRVLLGNESCTLTLSESTMNTLKCTVGPAMNKHFNMSIIISNGHGTTQYSTFSYVDPVITSISPKYGPMAGGTLLTLTGNYLNSGNSRHISIGGKTCTLKSVSNSILECYTPAQTISTEFAVKLKIDLANRETSIFSYREDPIVYEIHPTKSFISGGSTITGVGKNLNSVSVPRMVINVHEAGRNFTVACQHRSNSEIICCTTPSLQQLNLQLPLKTKAFFMLDGILSKYFDLIYVHNPVFKPFEKPVMISMGNENVLEIKGNDIDPEAVKGEVLKVGNKSCENIHLHSEAVLCTVPNDLLKLNSELNIEWKQAISSTVLGKVIVQPDQNFTASGAAWSHPQFEKGAAWSHPQFEKGAAWSHPQFEKGAAHHHHHH

SEQ ID NO: 14 - protein, 976 aa, synthetic construct
  REGION 1..976: note = Decoy Met mutation K842E-TAGs
MKAPAVLAPGILVLLFTLVQRSNGECKEALAKSEMNVNMKYQLPNFTAETPIQNVILHEHHIFLGATNYIYVLNEEDLQKVAEYKTGPVLEHPDCFPCQDCSSKANLSGGVWKDNINMALVVDTYYDDQLISCGSVNRGTCQRHVFPHNHTADIQSEVHCIFSPQIEEPSQCPDCVVSALGAKVLSSVKDRFINFFVGNTINSSYFPDHPLHSISVRRLKETKDGFMFLTDQSYIDVLPEFRDSYPIKYVHAFESNNFIYFLTVQRETLDAQTFHTRIIRFCSINSGLHSYMEMPLECILTEKRKKRSTKKEVFNILQAAYVSKPGAQLARQIGASLNDDILFGVFAQSKPDSAEPMDRSAMCAFPIKYVNDFFNKIVNKNNVRCLQHFYGPNHEHCFNRTLLRNSSGCEARRDEYRTEFTTALQRVDLFMGQFSEVLLTSISTFIKGDLTIANLGTSEGRFMQVVVSRSGPSTPHVNFLLDSHPVSPEVIVEHTLNQNGYTLVITGKKITKIPLNGLGCRHFQSCSQCLSAPPFVQCGWCHDKCVRSEECLSGTWTQQICLPAIYKVFPNSAPLEGGTRLTICGWDFGFRRNNKFDLKKTRVLLGNESCTLTLSESTMNTLKCTVGPAMNKHFNMSIIISNGHGTTQYSTFSYVDPVITSISPKYGPMAGGTLLTLTGNYLNSGNSRHISIGGKTCTLKSVSNSILECYTPAQTISTEFAVKLKIDLANRETSIFSYREDPIVYEIHPTKSFISGGSTITGVGKNLNSVSVPRMVINVHEAGRNFTVACQHRSNSEIICCTTPSLQQLNLQLPLKTKAFFMLDGILSKYFDLIYVHNPVFEPFEKPVMISMGNENVLEIKGNDIDPEAVKGEVLKVGNKSCENIHLHSEAVLCTVPNDLLKLNSELNIEWKQAISSTVLGKVIVQPDQNFTASGAAWSHPQFEKGAAWSHPQFEKGAAWSHPQFEKGAAHHHHHH

SEQ ID NO: 15 - protein, 131 aa, synthetic construct
  REGION 1..131: note = murine VL
METDTILLWVLLLWVPGSTGDIVLTQSPASLAVSLGQRATISCKASQSVDYDGGSYMSWFQQRPGQPPKLLISAASNLESGIPARFSGSGSGTDFTLNIHPVEEEDVATYYCQQSYEDPLTFGAGTKVEIK

SEQ ID NO: 16 - protein, 131 aa, synthetic construct
  REGION 1..131: note = murine VH
MGWSYIILFLVATATDGHSQVQLQQPGTELVKPGASVKLSCKASGYTFTSYWIHWVKQRPGQGLEWIGEINPSSGRTNYNEKFKNKVTVTVDKSSTTAYMQLSNLTSEDSAVYYCASRGYWGQGTTLTVSS

SEQ ID NO: 17 - protein, 131 aa, synthetic construct
  REGION 1..131: note = humanized VL-cl03G05
METDTILLWVLLLWVPGSTGDIVLTQSPASLAVSLGERATISCKASQSVDYDGGSYMSWFQQRPGQPPKLLIYAASNLESGVPDRFSGSGSGTDFTLNISPLEAEDVAVYYCQQSYEDPLTFGGGTKVEIK

SEQ ID NO: 18 - protein, 131 aa, synthetic construct
  REGION 1..131: note = humanized VH-cl03G05
MGWSYIILFLVATATDGHSQVQLVQPGTEVKKPGASVKLSCKASGYTFTSYWIHWVRQAPGQGLEWMGEINPSSGRTNYNEKFKNRVTITADKSTSTAYMQLSSLRSEDTAVYYCASRGYWGQGTTVTVSS

SEQ ID NO: 19 - protein, 131 aa, synthetic construct
  REGION 1..131: note = humanized VL-cl03F04
METDTILLWVLLLWVPGSTGDIVMTQSPDSLAVSLGERATINCKASQSVDYDGGSYMSWYQQKPGQPPKLLISAASNLESGVPDRFSGSGSGTDFTLTIHSLQAEDVAVYYCQQSYEDPLTFGAGTKVEIK

SEQ ID NO: 20 - protein, 131 aa, synthetic construct
  REGION 1..131: note = humanized VH-cl03F04
MGWSYIILFLVATATDGHSQVQLQQPGAEVKKPGSSVKLSCKASGYTFTSYWIHWVKQAPGQGLEWIGEINPSSGRTNYNEKFKNKVTITVDKSTSTAYMELSNLRSEDSAVYYCASRGYWGQGTTLTVSS

SEQ ID NO: 21 - protein, 131 aa, synthetic construct
  REGION 1..131: note = humanized VL-cl03H08
METDTILLWVLLLWVPGSTGDIVLTQSPASLAVSLGERATISCKASQSVDYDGGSYMSWYQQKPGQPPKLLIYAASNLESGVPDRFSGSGSGTDFTLNISSVQEEDVATYYCQQSYEDPLTFGAGTKVEIK

SEQ ID NO: 22 - protein, 131 aa, synthetic construct
  REGION 1..131: note = humanized VH-cl03H08
MGWSYIILFLVATATDGHSQVQLVQSGAEVKKPGSSVKLSCKASGYTFSSYWIHWVRQAPGQGLEWMGEINPSSGRTNYNEKFKNRVTITADKSTSTAYMELSNLRSEDSAVYYCASRGYWGQGTTLTVSS

SEQ ID NO: 23 - protein, 131 aa, synthetic construct
  REGION 1..131: note = humanized VL-cl04H08
METDTILLWVLLLWVPGSTGDIVLTQSPASLAVSLGERATINCKASQSVDYDGGSYMSWYQQRPGQPPKLLIYAASNLESGVPDRFSGSGSGTDFTLTIHSLQAEDVATYYCQQSYEDPLTFGGGTKVEIK

SEQ ID NO: 24 - protein, 131 aa, synthetic construct
  REGION 1..131: note = humanized VH-cl04H08
MGWSYIILFLVATATDGHSQVQLQQPGAEVKKPGSSVKLSCKASGYTFTSYWIHWVKQAPGQGLEWIGEINPSSGRTNYNEKFKNKVTITVDKSTSTAYMELSSLRSEDTAVYYCASRGYWGQGTTVTVSS

SEQ ID NO: 25 - DNA, 717 bp, synthetic construct
  misc_feature 1..717: note = humanized VL+CL-cl03E08 (nucleotides)
  source 1..717: mol_type = other DNA
atggagacagacacaatcctgctatgggtgctgctgctctgggttccaggctccactggtgatattgtgctgacccagagcccggacagcctggcagtgagtctgggtcaacgcgccaccattaactgcaaagccagccagagcgtggattatgacggcggtagctacatgagctggtttcagcagaaaccgggtcagccgccgaaactgctgatttatgccgccagcaatctggaaagcggcgttccggcccgttttagcggtagcggcagcggcaccgattttaccctgaccattagctcgctgcaggcggaggatgtggccacctattactgccagcagagctacgaagatccgctgacctttggcggcggtaccaaagtggagattaaacgaactgtggctgcaccatctgtcttcatcttcccgccatctgatgagcagttgaaatctggaactgcctctgttgtgtgcctgctgaataacttctatcccagagaggccaaagtacagtggaaggtggataacgccctccaatcgggtaactcccaggagagtgtcacagagcaggacagcaaggacagcacctacagcctcagcagcaccctgacgctgagcaaagcagactacgagaaacacaaagtctacgcctgcgaagtcacccatcagggcctgagctcgcccgtcacaaagagcttcaacaggggagagtgttaa

SEQ ID NO: 26 - DNA, 717 bp, synthetic construct
  misc_feature 1..717: note = humanized VL+CL-cl03G05 (nucleotides)
  source 1..717: mol_type = other DNA
atggagacagacacaatcctgctatgggtgctgctgctctgggttccaggctccactggtgacatcgtgctgacccagtcccctgcttccctcgctgtgtccctgggcgagagggctaccatctcctgtaaggcctcccagtccgtggactacgacggcggctcctacatgtcctggttccagcagaggcctggccagcctcccaagctgctgatctacgctgcctccaacctggagtccggcgtgcctgataggttcagcggatccggctccggcaccgacttcaccctgaatatctcccctctggaggctgaggacgtggccgtgtactactgccagcagtcctacgaggaccctctgaccttcggcggcggcaccaaggtggagatcaagagaactgtcgcagcaccttccgtctttattttcccaccatcagatgaacagctgaaatccggtactgccagtgtggtctgtctgctcaataatttctatccccgggaggctaaagtccagtggaaagtggataatgcccttcagtccggcaactcccaggagagcgtgaccgagcaggattctaaggactcaacatattcactgtcatctactctcaccctgtctaaggctgattacgaaaagcacaaggtgtacgcttgcgaagttactcatcagggcctctcttcccctgtgaccaagagtttcaaccggggcgagtgctaa

SEQ ID NO: 27 - DNA, 717 bp, synthetic construct
  misc_feature 1..717: note = humanized VL+CL-cl03F04 (nucleotides)
  source 1..717: mol_type = other DNA
atggagacagacacaatcctgctatgggtgctgctgctctgggttccaggctccactggtgacatcgtgatgacccagtcccctgactccctggctgtgtccctgggcgaaagggccaccatcaactgcaaggcctcccagtccgtggactacgacggcggctcctacatgtcctggtaccagcagaagcccggccagcctcccaagctgctgatctccgccgcttccaatctggagtccggcgtgcccgataggttttccggctccggctccggcaccgactttaccctgaccatccactccctgcaggccgaggacgtggctgtgtactactgccagcagtcctacgaggaccctctgaccttcggcgccggcaccaaggtggagatcaagagaactgtcgcagcaccttccgtctttattttcccaccatcagatgaacagctgaaatccggtactgccagtgtggtctgtctgctcaataatttctatccccgggaggctaaagtccagtggaaagtggataatgcccttcagtccggcaactcccaggagagcgtgaccgagcaggattctaaggactcaacatattcactgtcatctactctcaccctgtctaaggctgattacgaaaagcacaaggtgtacgcttgcgaagttactcatcagggcctctcttcccctgtgaccaagagtttcaaccggggcgagtgctaa

SEQ ID NO: 28 - DNA, 717 bp, synthetic construct
  misc_feature 1..717: note = humanized VL+CL-cl03H08 (nucleotides)
  source 1..717: mol_type = other DNA
atggagacagacacaatcctgctatgggtgctgctgctctgggttccaggctccactggtgacatcgtgctgacccagtcccctgcttccctggctgtgtccctgggcgagagggctaccatctcctgcaaggcctcccagtccgtggactacgacggcggctcctacatgtcctggtaccagcagaagcccggccagcctcccaagctgctgatctacgccgcctccaacctggagtccggcgtgcccgataggttctccggatccggctccggcaccgacttcaccctgaacatctcctccgtgcaggaggaggacgtggccacctactactgccagcagtcctatgaggaccccctgaccttcggcgctggcaccaaggtggagatcaagagaactgtcgcagcaccttccgtctttattttcccaccatcagatgaacagctgaaatccggtactgccagtgtggtctgtctgctcaataatttctatccccgggaggctaaagtccagtggaaagtggataatgcccttcagtccggcaactcccaggagagcgtgaccgagcaggattctaaggactcaacatattcactgtcatctactctcaccctgtctaaggctgattacgaaaagcacaaggtgtacgcttgcgaagttactcatcagggcctctcttcccctgtgaccaagagtttcaaccggggcgagtgctaa

SEQ ID NO: 29 - DNA, 717 bp, synthetic construct
  misc_feature 1..717: note = humanized VL+CL-cl04H08 (nucleotides)
  source 1..717: mol_type = other DNA
atggagacagacacaatcctgctatgggtgctgctgctctgggttccaggctccactggtgacatcgtgctgacccagtcccctgcttccctggctgtgtccctgggagagagggccaccatcaactgcaaggcctcccagtccgtggactacgacggcggctcctacatgtcctggtaccagcagaggcccggacagcctcccaagctgctgatctacgctgcctccaacctggagtccggcgtgcctgataggttttccggctccggctccggaaccgacttcaccctgaccatccactccctgcaggcggaggacgtggccacctactactgccagcagtcctacgaggaccccctgacattcggcggcggaaccaaggtggagatcaagagaactgtcgcagcaccttccgtctttattttcccaccatcagatgaacagctgaaatccggtactgccagtgtggtctgtctgctcaataatttctatccccgggaggctaaagtccagtggaaagtggataatgcccttcagtccggcaactcccaggagagcgtgaccgagcaggattctaaggactcaacatattcactgtcatctactctcaccctgtctaaggctgattacgaaaagcacaaggtgtacgcttgcgaagttactcatcagggcctctcttcccctgtgaccaagagtttcaaccggggcgagtgctaa

SEQ ID NO: 30 - DNA, 717 bp, synthetic construct
  misc_feature 1..717: note = chimeric VL+CL (nucleotides)
  source 1..717: mol_type = other DNA
atggagacagacacaatcctgctatgggtgctgctgctctgggttccaggctccactggtgacattgtgctgacccaatctccagcttctttggctgtgtctctagggcagagggccaccatctcctgcaaggccagccaaagtgttgattatgatggtggtagttatatgagttggttccaacagagaccaggacagccacccaaactcctcatctctgctgcatccaaccttgaatctggcatcccagccaggtttagtggcagtggctctgggacagacttcaccctcaatatccatcctgtggaggaggaggatgttgcaacctattactgtcagcaaagttatgaagacccgctcacgttcggtgctggtaccaaggtggagatcaaacgaactgtggctgcaccatctgtcttcatcttcccgccatctgatgagcagttgaaatctggaactgcctctgttgtgtgcctgctgaataacttctatcccagagaggccaaagtacagtggaaggtggataacgccctccaatcgggtaactcccaggagagtgtcacagagcaggacagcaaggacagcacctacagcctcagcagcaccctgacgctgagcaaagcagactacgagaaacacaaagtctacgcctgcgaagtcacccatcagggcctgagctcgcccgtcacaaagagcttcaacaggggagagtgttaa

SEQ ID NO: 31 - DNA, 1386 bp, synthetic construct
  misc_feature 1..1386: note = humanized VH+CH1+CH2+CH3-cl03E08, knob mutation, (nucleotides)
  source 1..1386: mol_type = other DNA
atgggatggagctatatcatcctctttttggtagcaacagctacagatggccactcccaggtgcagctgcagcagtcgggtgccgaagtgaaaaaaccgggtgctagtgtgaaactgagctgcaaagccagcggctataccttcaccagctactggatccactgggtgcgtcaggcgcctggccagggcctggaatggattggcgaaatcaatccgagcagcggtcgcaccaattacaatgaaaaatttaaaaatcgtgtgaccgttaccgtggataaaagcacctccaccgcctatatggagctgagcagcctgaccagcgaagatagcgccgtgtattattgcgccagccgcggttattggggccagggtaccaccctgaccgtgagcagcgctagcacgaagggcccatcggtcttccccctggcaccctcctccaagagcacctctgggggcacagcggccctgggctgcctggtcaaggactacttccccgaaccggtgacggtgtcgtggaactcaggcgccctgaccagcggcgtgcacaccttcccggctgtcctacagtcctcaggactctactccctcagcagcgtggtgaccgtgccctccagcagcttgggcacccagacctacatctgcaacgtgaatcacaagcccagcaacaccaaggtggacaagaaagttgagcccaaatcttgtgacaaaactcacacatgcccaccgtgcccagcacctgaactcctggggggaccgtcagtcttcctcttccccccaaaacccaaggacaccctcatgatctcccggacccctgaggtcacatgcgtggtggtggacgtgagccacgaagaccctgaggtcaagttcaactggtacgtggacggcgtggaggtgcataatgccaagacaaagccgcgggaggagcagtacaacagcacgtaccgtgtggtcagcgtcctcaccgtcctgcaccaggactggctgaatggcaaggagtacaagtgcaaggtctccaacaaagccctcccagcccccatcgagaaaaccatctccaaagccaaagggcagccccgagaaccacaggtgtacaccctgcccccatcccgggatgagctgaccaagaaccaggtcagcctgtggtgcctggtcaaaggcttctatcccagcgacatcgccgtggagtgggagagcaatgggcagccggagaacaactacaagaccacgcctcccgtgctggactccgacggctccttcttcctctacagcaagctcaccgtggacaagagcaggtggcagcaggggaacgtcttctcatgctccgtgatgcatgaggctctgcacaaccactacacgcagaagagcctctccctgtctccgggtaaatag

SEQ ID NO: 32 - DNA, 1386 bp, synthetic construct
  misc_feature 1..1386: note = humanized VH+CH1+CH2+CH3-cl03G05, knob mutation, (nucleotides)
  source 1..1386: mol_type = other DNA
atgggatggagctatatcatcctctttttggtagcaacagctacagatggccactcccaggtgcagctggtgcagcccggcacagaggtgaagaagcctggcgcctccgtgaagctgtcctgcaaggcctccggctacaccttcaccagctactggatccactgggtgaggcaggctcctggacagggcctggagtggatgggcgagatcaacccctcctccggcaggaccaactacaacgagaagttcaagaaccgggtgaccatcaccgccgacaagtccacctccaccgcctacatgcagctgtcctccctgaggtccgaggacaccgccgtgtactactgcgcctccaggggatattggggccagggcaccacagtgaccgtgagctccgctagcacgaagggcccatcggtcttccccctggcaccctcctccaagagcacctctgggggcacagcggccctgggctgcctggtcaaggactacttccccgaaccggtgacggtgtcgtggaactcaggcgccctgaccagcggcgtgcacaccttcccggctgtcctacagtcctcaggactctactccctcagcagcgtggtgaccgtgccctccagcagcttgggcacccagacctacatctgcaacgtgaatcacaagcccagcaacaccaaggtggacaagaaagttgagcccaaatcttgtgacaaaactcacacatgcccaccgtgcccagcacctgaactcctggggggaccgtcagtcttcctcttccccccaaaacccaaggacaccctcatgatctcccggacccctgaggtcacatgcgtggtggtggacgtgagccacgaagaccctgaggtcaagttcaactggtacgtggacggcgtggaggtgcataatgccaagacaaagccgcgggaggagcagtacaacagcacgtaccgtgtggtcagcgtcctcaccgtcctgcaccaggactggctgaatggcaaggagtacaagtgcaaggtctccaacaaagccctcccagcccccatcgagaaaaccatctccaaagccaaagggcagccccgagaaccacaggtgtacaccctgcccccatcccgggatgagctgaccaagaaccaggtcagcctgtggtgcctggtcaaaggcttctatcccagcgacatcgccgtggagtgggagagcaatgggcagccggagaacaactacaagaccacgcctcccgtgctggactccgacggctccttcttcctctacagcaagctcaccgtggacaagagcaggtggcagcaggggaacgtcttctcatgctccgtgatgcatgaggctctgcacaaccactacacgcagaagagcctctccctgtctccgggtaaatag

SEQ ID NO: 33 - DNA, 1386 bp, synthetic construct
  misc_feature 1..1386: note = humanized VH+CH1+CH2+CH3-cl03F04, knob mutation (nucleotides)
  source 1..1386: mol_type = other DNA
atgggatggagctatatcatcctctttttggtagcaacagctacagatggccactcccaggtgcagctgcagcagcccggagccgaagtgaagaagcccggctccagcgtgaagctgtcctgcaaggcctccggctacaccttcacctcctactggatccactgggtgaagcaggctcctggacagggcctggagtggatcggcgagatcaacccctcctccggccggaccaactacaacgagaagttcaagaacaaggtgaccatcaccgtggacaagtccacctccaccgcctacatggagctgtccaacctgcggtccgaggactccgccgtgtactactgtgcctccaggggctattggggccagggcacaaccctgaccgtgtcctccgctagcacgaagggcccatcggtcttccccctggcaccctcctccaagagcacctctgggggcacagcggccctgggctgcctggtcaaggactacttccccgaaccggtgacggtgtcgtggaactcaggcgccctgaccagcggcgtgcacaccttcccggctgtcctacagtcctcaggactctactccctcagcagcgtggtgaccgtgccctccagcagcttgggcacccagacctacatctgcaacgtgaatcacaagcccagcaacaccaaggtggacaagaaagttgagcccaaatcttgtgacaaaactcacacatgcccaccgtgcccagcacctgaactcctggggggaccgtcagtcttcctcttccccccaaaacccaaggacaccctcatgatctcccggacccctgaggtcacatgcgtggtggtggacgtgagccacgaagaccctgaggtcaagttcaactggtacgtggacggcgtggaggtgcataatgccaagacaaagccgcgggaggagcagtacaacagcacgtaccgtgtggtcagcgtcctcaccgtcctgcaccaggactggctgaatggcaaggagtacaagtgcaaggtctccaacaaagccctcccagcccccatcgagaaaaccatctccaaagccaaagggcagccccgagaaccacaggtgtacaccctgcccccatcccgggatgagctgaccaagaaccaggtcagcctgtggtgcctggtcaaaggcttctatcccagcgacatcgccgtggagtgggagagcaatgggcagccggagaacaactacaagaccacgcctcccgtgctggactccgacggctccttcttcctctacagcaagctcaccgtggacaagagcaggtggcagcaggggaacgtcttctcatgctccgtgatgcatgaggctctgcacaaccactacacgcagaagagcctctccctgtctccgggtaaatag

SEQ ID NO: 34 - DNA, 1386 bp, synthetic construct
  misc_feature 1..1386: note = humanized VH+CH1+CH2+CH3-cl03H08, knob mutation, (nucleotides)
  source 1..1386: mol_type = other DNA
atgggatggagctatatcatcctctttttggtagcaacagctacagatggccactcccaggtgcagctggtgcagtccggcgccgaagtgaagaagcccggctcctccgtgaagctgagctgcaaggcctccggctacaccttctcctcctactggatccactgggtgaggcaggctcctggacagggcctggagtggatgggcgagatcaacccctcctccggcaggaccaactacaacgagaagttcaagaaccgggtgaccatcaccgccgacaagtccacctccaccgcctacatggagctgtccaacctgaggtccgaggactccgccgtgtactactgcgcctccaggggatattggggccagggcaccaccctgacagtgtcctccgctagcacgaagggcccatcggtcttccccctggcaccctcctccaagagcacctctgggggcacagcggccctgggctgcctggtcaaggactacttccccgaaccggtgacggtgtcgtggaactcaggcgccctgaccagcggcgtgcacaccttcccggctgtcctacagtcctcaggactctactccctcagcagcgtggtgaccgtgccctccagcagcttgggcacccagacctacatctgcaacgtgaatcacaagcccagcaacaccaaggtggacaagaaagttgagcccaaatcttgtgacaaaactcacacatgcccaccgtgcccagcacctgaactcctggggggaccgtcagtcttcctcttccccccaaaacccaaggacaccctcatgatctcccggacccctgaggtcacatgcgtggtggtggacgtgagccacgaagaccctgaggtcaagttcaactggtacgtggacggcgtggaggtgcataatgccaagacaaagccgcgggaggagcagtacaacagcacgtaccgtgtggtcagcgtcctcaccgtcctgcaccaggactggctgaatggcaaggagtacaagtgcaaggtctccaacaaagccctcccagcccccatcgagaaaaccatctccaaagccaaagggcagccccgagaaccacaggtgtacaccctgcccccatcccgggatgagctgaccaagaaccaggtcagcctgtggtgcctggtcaaaggcttctatcccagcgacatcgccgtggagtgggagagcaatgggcagccggagaacaactacaagaccacgcctcccgtgctggactccgacggctccttcttcctctacagcaagctcaccgtggacaagagcaggtggcagcaggggaacgtcttctcatgctccgtgatgcatgaggctctgcacaaccactacacgcagaagagcctctccctgtctccgggtaaatag

SEQ ID NO: 35 - DNA, 1386 bp, synthetic construct
  misc_feature 1..1386: note = humanized VH+CH1+CH2+CH3-cl04H08, knob mutation, (nucleotides)
  source 1..1386: mol_type = other DNA
atgggatggagctatatcatcctctttttggtagcaacagctacagatggccactcccaggtgcagctgcagcagcctggagccgaggtgaagaagcccggctcctccgtgaagctgtcctgcaaggcctccggctacaccttcacctcctactggatccactgggtgaagcaggcccctggacagggcctggagtggatcggcgagatcaacccctcctccggcaggaccaactacaacgagaagttcaagaacaaggtgaccatcaccgtggacaagtccacctccaccgcctacatggagctgtcctccctgaggtccgaggacaccgccgtgtactactgtgcctccaggggctattggggccagggcacaaccgtgaccgtgtcctccgctagcacgaagggcccatcggtcttccccctggcaccctcctccaagagcacctctgggggcacagcggccctgggctgcctggtcaaggactacttccccgaaccggtgacggtgtcgtggaactcaggcgccctgaccagcggcgtgcacaccttcccggctgtcctacagtcctcaggactctactccctcagcagcgtggtgaccgtgccctccagcagcttgggcacccagacctacatctgcaacgtgaatcacaagcccagcaacaccaaggtggacaagaaagttgagcccaaatcttgtgacaaaactcacacatgcccaccgtgcccagcacctgaactcctggggggaccgtcagtcttcctcttccccccaaaacccaaggacaccctcatgatctcccggacccctgaggtcacatgcgtggtggtggacgtgagccacgaagaccctgaggtcaagttcaactggtacgtggacggcgtggaggtgcataatgccaagacaaagccgcgggaggagcagtacaacagcacgtaccgtgtggtcagcgtcctcaccgtcctgcaccaggactggctgaatggcaaggagtacaagtgcaaggtctccaacaaagccctcccagcccccatcgagaaaaccatctccaaagccaaagggcagccccgagaaccacaggtgtacaccctgcccccatcccgggatgagctgaccaagaaccaggtcagcctgtggtgcctggtcaaaggcttctatcccagcgacatcgccgtggagtgggagagcaatgggcagccggagaacaactacaagaccacgcctcccgtgctggactccgacggctccttcttcctctacagcaagctcaccgtggacaagagcaggtggcagcaggggaacgtcttctcatgctccgtgatgcatgaggctctgcacaaccactacacgcagaagagcctctccctgtctccgggtaaatag

SEQ ID NO: 36 - DNA, 1386 bp, synthetic construct
  misc_feature 1..1386: note = chimeric VH+CH1+CH2+CH3, knob mutation, (nucleotides)
  source 1..1386: mol_type = other DNA
atgggatggagctatatcatcctctttttggtagcaacagctacagatggccactcccaggtccaactgcaacagcctgggactgaactggtgaagcctggggcttcagtgaagctgtcctgcaaggcttctggctacaccttcaccagttactggatacactgggtgaagcagaggcctggacaaggccttgagtggattggagagattaatcctagcagcggtcgtactaactacaacgagaaattcaagaacaaggtcacagtgactgtagacaaatcttccaccacagcctacatgcaactcagcaacctgacatctgaggactctgcggtctattactgtgcaagtaggggctactggggccaaggcaccactctcacagtctcctcagctagcacgaagggcccatcggtcttccccctggcaccctcctccaagagcacctctgggggcacagcggccctgggctgcctggtcaaggactacttccccgaaccggtgacggtgtcgtggaactcaggcgccctgaccagcggcgtgcacaccttcccggctgtcctacagtcctcaggactctactccctcagcagcgtggtgaccgtgccctccagcagcttgggcacccagacctacatctgcaacgtgaatcacaagcccagcaacaccaaggtggacaagaaagttgagcccaaatcttgtgacaaaactcacacatgcccaccgtgcccagcacctgaactcctggggggaccgtcagtcttcctcttccccccaaaacccaaggacaccctcatgatctcccggacccctgaggtcacatgcgtggtggtggacgtgagccacgaagaccctgaggtcaagttcaactggtacgtggacggcgtggaggtgcataatgccaagacaaagccgcgggaggagcagtacaacagcacgtaccgtgtggtcagcgtcctcaccgtcctgcaccaggactggctgaatggcaaggagtacaagtgcaaggtctccaacaaagccctcccagcccccatcgagaaaaccatctccaaagccaaagggcagccccgagaaccacaggtgtacaccctgcccccatcccgggatgagctgaccaagaaccaggtcagcctgtggtgcctggtcaaaggcttctatcccagcgacatcgccgtggagtgggagagcaatgggcagccggagaacaactacaagaccacgcctcccgtgctggactccgacggctccttcttcctctacagcaagctcaccgtggacaagagcaggtggcagcaggggaacgtcttctcatgctccgtgatgcatgaggctctgcacaaccactacacgcagaagagcctctccctgtctccgggtaaatag

SEQ ID NO: 37 - DNA, 741 bp, synthetic construct
  misc_feature 1..741: note = human CH2+CH3, Hole mutations, (nucleotides)
  source 1..741: mol_type = other DNA
atgggatggagctatatcatcctctttttggtagcaacagctacagatggccactccgacaaaactcacacatgcccaccgtgcccagcacctgaactcctggggggaccgtcagtcttcctcttccccccaaaacccaaggacaccctcatgatctcccggacccctgaggtcacatgcgtggtggtggacgtgagccacgaagaccctgaggtcaagttcaactggtacgtggacggcgtggaggtgcataatgccaagacaaagccgcgggaggagcagtacaacagcacgtaccgtgtggtcagcgtcctcaccgtcctgcaccaggactggctgaatggcaaggagtacaagtgcaaggtctccaacaaagccctcccagcccccatcgagaaaaccatctccaaagccaaagggcagccccgagaaccacaggtgtacaccctgcccccatcccgggatgagctgaccaagaaccaggtcagcctgagttgcgcggtcaaaggcttctatcccagcgacatcgccgtggagtgggagagcaatgggcagccggagaacaactacaagaccacgcctcccgtgctggactccgacggctccttcttcctcgtcagcaagctcaccgtggacaagagcaggtggcagcaggggaacgtcttctcatgctccgtgatgcatgaggctctgcacaaccactacacgcagaagagcctctccctgtctccgggtaaatag

SEQ ID NO: 38 - DNA, 18 bp, synthetic construct
  misc_feature 1..18: note = His-TAG (nucleotide)
  source 1..18: mol_type = other DNA
caccatcaccatcaccat

SEQ ID NO: 39 - protein, 6 aa, synthetic construct
  REGION 1..6: note = His-TAG
HHHHHH

SEQ ID NO: 40 - DNA, 108 bp, synthetic construct
  misc_feature 1..108: note = Strep-TAG (nucleotide)
  source 1..108: mol_type = other DNA
ggtgccgcatggagccacccccagttcgaaaaaggggccgcatggagccacccccagttcgaaaaaggggccgcatggagccacccccagttcgaaaaaggggccgca

SEQ ID NO: 41 - protein, 36 aa, synthetic construct
  REGION 1..36: note = Strep-TAG
GAAWSHPQFEKGAAWSHPQFEKGAAWSHPQFEKGAA

SEQ ID NO: 42 - DNA, 39 bp, synthetic construct
  misc_feature 1..39: note = K842E sense nucleotide
  source 1..39: mol_type = other DNA
gtacataatcctgtgtttgagccttttgaaaagccagtg

SEQ ID NO: 43 - DNA, 39 bp, synthetic construct
  misc_feature 1..39: note = K842E antisense nucleotide
  source 1..39: mol_type = other DNA
cactggcttttcaaaaggctcaaacacaggattatgtac